European Patent Application EP 4 502 161 A1, published February 5, 2025. Title: ALPHA-AMYLASE VARIANT. Applicant: KAO CORPORATION. The sequence listing filed with the application follows.

SEQUENCE LISTING (26 sequences)

SEQ ID NO: 1 - protein, 485 aa, Bacillus sp. YR288
AAQNGTMMQYFEWYVPNDGQHWNRLRNDAAYLKSIGVSAIWTPPAYKGTSQNDVGYGAYDLYDLGEFNQKGTIRTKYGTKAELKSAVSTLKSNGIQVYGDVVMNHKGGADYTENVTAVEVNPSNRNQETSDEYTIQAWTGFNFPGRGTTHSPFKWQWYHFDGTDWDQSRNASRIFKFRGTGKAWDWEVSSENGNYDYLMYADLDFDHPDVRNEMKNWGVWYANEVGLDGFRLDAVKHIKHSYLGDWVNHVRTKTGKEMFTVAEYWQNDVNAINNYLAKVNYNHSVFDAPLHYNFHYASQSGGNYDMRNLLNGTVVAAHPTKAVTLVENHDSQPGQSLESVVQPWFKPLAYAFILTRAEGYPSIFYGDMYGTKGNSSYEIPALKTKIEPLLKARKDYAYGTQHNYMDHWDVIGWTREGDSTKEKSGLATLVTDGAGGSKWMYVGKQNAGEVWYDITGNRTDKITINTDGWGNFQVNGGSVSVYVQQ

SEQ ID NO: 2 - protein, 483 aa, synthetic construct
AAQNGTMMQYFEWYVPNDGQHWNRLRNDAAYLKSIGVSAIWTPPAYKGTSQNDVGYGAYDLYDLGEFNQKGTIRTKYGTKAELKSAVSTLKSNGIQVYGDVVMNHKGGADYTENVTAVEVNPSNRNQETSDEYTIQAWTGFNFPGRGTTHSPFKWQWYHFDGTDWDQSRNASRIFKFGGKAWDWEVSSENGNYDYLMYADLDFDHPDVRNEMKNWGVWYANEVGLDGFRLDAVKHIKHSYLGDWVNHVRTKTGKEMFTVAEYWQNDVNAINNYLAKVNYNHSVFDAPLHYNFHYASQSGGNYDMRNLLNGTVVAAHPTKAVTLVENHDSQPGQSLESVVQPWFKPLAYAFILTRAEGYPSIFYGDMYGTKGNSSYEIPALKTKIEPLLKARKDYAYGTQHNYMDHWDVIGWTREGDSTKEKSGLATLVTDGAGGSKWMYVGKQNAGEVWYDITGNRTDKITINTDGWGNFQVNGGSVSVYVQQ

SEQ ID NO: 3 - DNA, 1458 bp, synthetic construct
  source 1..1458: mol_type = other DNA
  CDS 1..1455
catcatgatggcacaaacggaacaatcatgcaatactttgaatggaatgtcccgaacgatggccaacattggaaccgcttacataataacgctcagaatctgaaaaacgcaggcatcacagcgatttggatcccgccggcttggaaaggaacatcacaaaatgatgtcggctatggagcctatgatctgtatgatcttggcgaatttaaccagaaaggaacagttagaacaaaatatggaacaaaagctgaacttgaaagagccattcgcagcttaaaagcaaatggcatccaagtttatggagatgttgtgatgaaccataaaggcggagctgattttacagaacgcgtgcaggccgtcgaagttaatccgcaaaatagaaaccaggaagtcagcggcacatatcaaattgaagcgtggacaggatttaattttccgggccgcggaaaccagcattcaagctttaaatggagatggtatcattttgatggcacagattgggatcaatctagacagctggcaaatcgcatctataaatttagaggcgatggaaaagcgtgggattgggaagtggatacagaaaacggaaactacgattacctgatgtacgctgatgtcgatatggatcatccggaagttattaatgaactgaaccgctggggcgtttggtacgctaacacacttaacctggatggatttagattagatgccgtgaaacatatcaaattttcttttatgcgcgattggctgggccatgttagaggccagacaggaaaaaatctttttgcagtggcggaatattggaaaaacgatttaggagccctggaaaactacctttcaaaaacaaactggacaatgagcgcatttgatgtcccgcttcattacaacctgtaccaagcgtcaaactcttcaggcaactatgatatgcgcaatctgcttaacggaacactggttcagagacatccgtctcatgcagtgacatttgtcgataaccatgatacacaaccgggcgaagcgcttgaatcatttgtgcagggatggtttaaaccgctggcttatgccacaattcttacaagagaacaaggctatccgcaggtcttttatggcgattattatggaattccgtcagatggagttccgagctatcgccaacagatcgatccgttactgaaagcaagacaacagtatgcgtatggcacacaacatgattatcttgataatcaggatgtgatcggctggacacgcgaaggagattctgcacatgcgggctcaggattagctacagtcatgagcgatggcccgggcggatctaaaacaatgtatgtgggcacagctcatgccggacaagtctttaaagatatcacaggaaacagaacagatacagttacaatcaacagcgccggcaacggaacatttccgtgcaacggcggaagcgtttctatttgggtgaaacagtaa

SEQ ID NO: 4 - protein, 485 aa, synthetic construct
HHDGTNGTIMQYFEWNVPNDGQHWNRLHNNAQNLKNAGITAIWIPPAWKGTSQNDVGYGAYDLYDLGEFNQKGTVRTKYGTKAELERAIRSLKANGIQVYGDVVMNHKGGADFTERVQAVEVNPQNRNQEVSGTYQIEAWTGFNFPGRGNQHSSFKWRWYHFDGTDWDQSRQLANRIYKFRGDGKAWDWEVDTENGNYDYLMYADVDMDHPEVINELNRWGVWYANTLNLDGFRLDAVKHIKFSFMRDWLGHVRGQTGKNLFAVAEYWKNDLGALENYLSKTNWTMSAFDVPLHYNLYQASNSSGNYDMRNLLNGTLVQRHPSHAVTFVDNHDTQPGEALESFVQGWFKPLAYATILTREQGYPQVFYGDYYGIPSDGVPSYRQQIDPLLKARQQYAYGTQHDYLDNQDVIGWTREGDSAHAGSGLATVMSDGPGGSKTMYVGTAHAGQVFKDITGNRTDTVTINSAGNGTFPCNGGSVSIWVKQ

SEQ ID NO: 5 - DNA, 1458 bp, synthetic construct
  source 1..1458: mol_type = other DNA
  CDS 1..1455: note = Codon-optimized oligonucleotide
gccgccactaatgggacgatgatgcagtactttgaatggtacgttccgaatgatggccaacagtggaacaggctgagaacagacgcaccgtacttatcaagcgttggcattacggctgtctggacgccaccggcgtataagggtacttcacaagcggatgttggatacggaccatatgacttgtacgatttaggggagtttaaccagaaagggacagtacgcaccaaatatggaacaaaaggcgaactgaaaagcgccgtcaatacgctgcattccaatggaattcaggtctatggcgatgtggttatgaaccataaagcaggagcggactatactgagaatgttactgcagtggaagtgaatccatccaatcgaaaccaggaaacttcaggagaatacaacatacaggcgtggaccggctttaacttcccaggccgtggaacgacatatagcaactttaaatggcaatggtttcactttgatggtacagattgggatcaaagccgatcactctccaggatcttcaagtttcgcggtacaggcaaagcttgggattgggaggtgtcgtctgaaaacggcaattacgattaccttatgtatgcagatatcgactatgaccatcctgacgtcgttaatgagatgaagaaatggggagtatggtacgctaatgaagtaggtttagatgggtatcggttggatgccgtcaaacacatcaaattcagctttctcaaagattgggtcgataacgcgagagcagcaaccgggaaggagatgtttacagtgggtgaatattggcaaaatgacttaggagctcttaacaactatttggcgaaagtcaactataatcagtctctgtttgatgctccgcttcattacaacttctatgcggctagtacaggaggtgggtattatgacatgcgcaacattctgaataatacgctggttgcgtctaatcccacaaaagctgttaccctggtagaaaatcatgacacacaaccgggccagtctttggaatccacagtgcaaccgtggttcaaacctctcgcatatgcttttatcttaacacgctctggcggatatccctcagtgttctacggggatatgtatggcacaaagggaacgacgacacgggaaattcctgcactgaaatcgaagattgaacctcttcttaaggcacggaaagactatgcctatggcactcaacgtgattatattgacaaccctgacgtcattggctggacaagagagggagattcgaccaaagcgaaaagcggattagcaacggtaatcactgatggcccgggtggatctaagcgtatgtatgtcggtacgtcaaatgccggggaaatctggtacgatcttaccggcaatagaaccgataaaattacgataggcagtgatggttatgccacatttccggttaatggaggctcagtgagtgtatgggtgcaacagtaa

SEQ ID NO: 6 - protein, 485 aa, Cytophaga sp.
AATNGTMMQYFEWYVPNDGQQWNRLRTDAPYLSSVGITAVWTPPAYKGTSQADVGYGPYDLYDLGEFNQKGTVRTKYGTKGELKSAVNTLHSNGIQVYGDVVMNHKAGADYTENVTAVEVNPSNRNQETSGEYNIQAWTGFNFPGRGTTYSNFKWQWFHFDGTDWDQSRSLSRIFKFRGTGKAWDWEVSSENGNYDYLMYADIDYDHPDVVNEMKKWGVWYANEVGLDGYRLDAVKHIKFSFLKDWVDNARAATGKEMFTVGEYWQNDLGALNNYLAKVNYNQSLFDAPLHYNFYAASTGGGYYDMRNILNNTLVASNPTKAVTLVENHDTQPGQSLESTVQPWFKPLAYAFILTRSGGYPSVFYGDMYGTKGTTTREIPALKSKIEPLLKARKDYAYGTQRDYIDNPDVIGWTREGDSTKAKSGLATVITDGPGGSKRMYVGTSNAGEIWYDLTGNRTDKITIGSDGYATFPVNGGSVSVWVQQ

SEQ ID NO: 7 - DNA, 1458 bp, synthetic construct
  source 1..1458: mol_type = other DNA
  CDS 1..1455: note = Codon-optimized oligonucleotide
catcataatggaacaaacggcacaatgatgcaatactttgaatggtatttaccgaacgatggaaaccattggaatagattacgcagcgatgcgtctaacctgaaagataaaggaatttcagctgtttggatcccgccggcatggaaaggagctagccaaaatgatgtgggctatggagcgtacgatctttacgatctgggagaatttaaccagaaaggcacaattcgcacaaaatatggcacaagaaatcaacttcaggcagcggtgaacgctttaaaatcaaatggaatccaagtctatggcgatgttgtgatgaatcataaaggcggagctgatgccacagaaatggtccgcgccgttgaagtgaacccgaataacagaaatcaggaagttagcggagaatacacaatcgaagcatggacaaaatttgattttccgggccgcggaaacacacattctaactttaaatggagatggtaccattttgatggcgttgattgggatcagtcaagaaaactgaacaaccgcatctacaaatttagaggcgatggaaaaggctgggattgggaagtggatacagaaaacggaaactacgattacctgatgtatgccgatatcgatatggatcatccggaagtcgttaacgaacttcgcaattggggcgtgtggtatacaaatacactgggacttgatggctttagaattgatgcggtcaaacatatcaaatatagctttacacgcgattggattaaccatgttagatctgcgacaggaaaaaatatgtttgcagtggcggaattttggaaaaatgatctgggcgctatcgaaaactaccttaacaaaacaaactggaaccattctgtctttgatgttccgctgcattacaacctttacaacgcgtcaaaaagcggcggaaactatgatatgcgccaaatttttaatggaacagtggtccagagacatccgatgcatgccgtgacatttgtcgataatcatgattctcaaccggaagaagcactggaatcatttgttgaagaatggtttaaaccgctggcttatgccttaacactgacacgcgaacagggatatccgagcgtgttttatggagattattatggcatcccgacacatggcgtcccggctatgaaatctaaaattgatccgatccttgaagctcgccaaaaatatgcctatggcagacagaacgattacctggatcatcataacatcatcggatggacaagagaaggcaacacagcacatccgaattcaggacttgcgacaattatgagcgatggcgctggcggaaacaaatggatgtttgtcggacgcaataaagcaggccaagtttggacagatattacaggaaacagagccggaacagtcacaatcaatgcagatggatggggcaactttagcgttaatggcggctcagtttcaatctgggtgaataaataa

SEQ ID NO: 8 - protein, 485 aa, Bacillus sp. DSM12649
HHNGTNGTMMQYFEWYLPNDGNHWNRLRSDASNLKDKGISAVWIPPAWKGASQNDVGYGAYDLYDLGEFNQKGTIRTKYGTRNQLQAAVNALKSNGIQVYGDVVMNHKGGADATEMVRAVEVNPNNRNQEVSGEYTIEAWTKFDFPGRGNTHSNFKWRWYHFDGVDWDQSRKLNNRIYKFRGDGKGWDWEVDTENGNYDYLMYADIDMDHPEVVNELRNWGVWYTNTLGLDGFRIDAVKHIKYSFTRDWINHVRSATGKNMFAVAEFWKNDLGAIENYLNKTNWNHSVFDVPLHYNLYNASKSGGNYDMRQIFNGTVVQRHPMHAVTFVDNHDSQPEEALESFVEEWFKPLAYALTLTREQGYPSVFYGDYYGIPTHGVPAMKSKIDPILEARQKYAYGRQNDYLDHHNIIGWTREGNTAHPNSGLATIMSDGAGGNKWMFVGRNKAGQVWTDITGNRAGTVTINADGWGNFSVNGGSVSIWVNK

SEQ ID NO: 9 - DNA, 1458 bp, synthetic construct
  source 1..1458: mol_type = other DNA
  CDS 1..1455: note = Codon-optimized oligonucleotide
catcataatggcacaaacggaacaatgatgcaatattttgaatggcatctgccgaatgatggcaaccattggaatagactgcgcgatgatgcttctaaccttagaaatcgcggcattacagctatttggatcccgccggcctggaaaggaacatcacagaatgatgtcggctatggagcctatgatctgtatgatcttggcgaatttaaccaaaaaggaacagttcgcacaaaatatggaacaagatcacagttagaaagcgctatccatgccctgaaaaataacggcgttcaagtgtatggagatgttgtgatgaatcataaaggcggagcagatgcgacagaaaacgtgcttgctgtcgaagttaatccgaataaccgcaaccaggaaatttcaggcgattatacaatcgaagcctggacaaaatttgattttccgggccgcggaaacacatactcagattttaaatggagatggtaccattttgatggagtcgattgggatcaaagcagacaatttcagaaccgcatctacaaatttagaggcgatggaaaagcttgggattgggaagttgatagcgaaaatggcaactatgattatctgatgtatgccgatgtggatatggatcatccggaagtcgttaatgaacttagacgctggggcgaatggtacacaaacacactgaacctggatggatttagaatcgatgcggttaaacatatcaaatacagctttacacgcgattggttaacacatgttagaaatgcaacaggcaaagaaatgtttgctgtggccgaattttggaaaaacgatttaggagcgctggaaaactacctgaacaaaacaaactggaaccattctgtgtttgatgtcccgcttcattacaacctgtacaacgcatcaaacagcggcggaaattatgatatggcgaaactgcttaacggcacagtggtccaaaaacatccgatgcatgcagttacatttgtggataatcatgattctcaaccgggagaaagccttgaatcttttgtgcaggaatggtttaaaccgttagcatatgcgcttattttaacacgcgaacagggctatccgagcgtgttttatggcgattattatggaatcccgacacattctgtcccggcaatgaaagcgaaaattgatccgatccttgaagcacgccaaaattttgcgtatggaacacagcatgattactttgatcatcataacatcatcggctggacaagagaaggaaatacaacacatccgaactctggcttagcaacaattatgtcagatggaccgggcggagaaaaatggatgtatgtgggccaaaataaagcgggacaggtctggcatgatattacaggcaataaaccgggaacagtcacaatcaacgctgatggatgggccaattttagcgttaacggcggatctgtctcaatctgggttaaaagataa

SEQ ID NO: 10 - protein, 485 aa, Bacillus sp. SP722
HHNGTNGTMMQYFEWHLPNDGNHWNRLRDDASNLRNRGITAIWIPPAWKGTSQNDVGYGAYDLYDLGEFNQKGTVRTKYGTRSQLESAIHALKNNGVQVYGDVVMNHKGGADATENVLAVEVNPNNRNQEISGDYTIEAWTKFDFPGRGNTYSDFKWRWYHFDGVDWDQSRQFQNRIYKFRGDGKAWDWEVDSENGNYDYLMYADVDMDHPEVVNELRRWGEWYTNTLNLDGFRIDAVKHIKYSFTRDWLTHVRNATGKEMFAVAEFWKNDLGALENYLNKTNWNHSVFDVPLHYNLYNASNSGGNYDMAKLLNGTVVQKHPMHAVTFVDNHDSQPGESLESFVQEWFKPLAYALILTREQGYPSVFYGDYYGIPTHSVPAMKAKIDPILEARQNFAYGTQHDYFDHHNIIGWTREGNTTHPNSGLATIMSDGPGGEKWMYVGQNKAGQVWHDITGNKPGTVTINADGWANFSVNGGSVSIWVKR

SEQ ID NO: 11 - DNA, 1458 bp, synthetic construct
  source 1..1458: mol_type = other DNA
  CDS 1..1455: note = Codon-optimized oligonucleotide
catcataatggcacaaacggaacaatgatgcagtattttgaatggcatttaccgaatgatggcaaccattggaatagactgcgcgatgatgcagcgaatcttaaaagcaaaggcattacagctgtttggatcccgccggcctggaaaggaacatctcaaaacgatgtgggctatggagcttacgatctgtacgatctgggcgaatttaatcagaaaggaacagtcagaacaaaatatggcacacgctctcaattacagggagccgtgacatcactgaaaaataacggcattcaagtctatggagatgttgtgatgaatcataaaggcggagcagatggcacagaaatggttaatgcggttgaagtgaacagaagcaatcgcaaccaggaaatttctggagaatatacaatcgaagcatggacaaaatttgattttccgggcagaggaaatacacattcaaactttaaatggcgctggtatcattttgatggcacagattgggatcaaagcagacaactgcagaacaaaatctacaaatttcgcggcacaggaaaagcttgggattgggaagtggatatcgaaaacggaaactacgattacctgatgtacgccgatattgatatggatcatccggaagtcatcaatgaactgagaaactggggcgtttggtacacaaacacacttaacctggatggatttcgcattgatgcggtcaaacatatcaaatactcatacacaagagattggctgacacatgttcgcaatacaacaggcaaaccgatgtttgcagtggcggaattttggaaaaacgatcttgctgccatcgaaaactacctgaacaaaacatcatggaatcatagcgtctttgatgttccgcttcattacaacctgtacaacgcttctaactcaggcggatattttgatatgagaaacatccttaacggctctgtcgttcagaaacatccgatccatgcagtgacatttgtcgataatcatgattcacaaccgggagaagcgctggaatcttttgtgcagtcatggtttaaaccgcttgcttatgccctgattcttacacgcgaacaaggctatccgagcgtgttttatggcgattattatggaattccgacacatggagtcccgagcatgaaatctaaaatcgatccgttactgcaagcaagacagacatatgcgtatggaacacagcatgattactttgatcatcatgatatcatcggctggacacgcgaaggagattcaagccatccgaattcaggccttgcaacaatcatgagcgatggaccgggcggaaacaaatggatgtatgttggcaaacataaagcgggacaagtgtggagagatattacaggcaatcgcagcggaacagtcacaatcaacgctgatggctggggaaattttacagttaacggcggagccgtctctgtttgggtgaaacagtaa

SEQ ID NO: 12 - protein, 485 aa, Bacillus sp. KSM-1378
HHNGTNGTMMQYFEWHLPNDGNHWNRLRDDAANLKSKGITAVWIPPAWKGTSQNDVGYGAYDLYDLGEFNQKGTVRTKYGTRSQLQGAVTSLKNNGIQVYGDVVMNHKGGADGTEMVNAVEVNRSNRNQEISGEYTIEAWTKFDFPGRGNTHSNFKWRWYHFDGTDWDQSRQLQNKIYKFRGTGKAWDWEVDIENGNYDYLMYADIDMDHPEVINELRNWGVWYTNTLNLDGFRIDAVKHIKYSYTRDWLTHVRNTTGKPMFAVAEFWKNDLAAIENYLNKTSWNHSVFDVPLHYNLYNASNSGGYFDMRNILNGSVVQKHPIHAVTFVDNHDSQPGEALESFVQSWFKPLAYALILTREQGYPSVFYGDYYGIPTHGVPSMKSKIDPLLQARQTYAYGTQHDYFDHHDIIGWTREGDSSHPNSGLATIMSDGPGGNKWMYVGKHKAGQVWRDITGNRSGTVTINADGWGNFTVNGGAVSVWVKQ

SEQ ID NO: 13 - DNA, 29 bp, synthetic construct
  source 1..29: mol_type = other DNA
taatctattaaactagttatagggttatc

SEQ ID NO: 14 - DNA, 18 bp, synthetic construct
  source 1..18: mol_type = other DNA
tgctgcaagagctgccgg

SEQ ID NO: 15 - DNA, 33 bp, synthetic construct
  source 1..33: mol_type = other DNA
gcagctcttgcagcacatcatgatggcacaaac

SEQ ID NO: 16 - DNA, 36 bp, synthetic construct
  source 1..36: mol_type = other DNA
tagtttaatagattactgtttcacccaaatagaaac

SEQ ID NO: 17 - DNA, 35 bp, synthetic construct
  source 1..35: mol_type = other DNA
cgcatctataaatttggcggaaaagcgtgggattg

SEQ ID NO: 18 - DNA, 24 bp, synthetic construct
  source 1..24: mol_type = other DNA
aaatttatagatgcgatttgccag

SEQ ID NO: 19 - DNA, 35 bp, synthetic construct
  source 1..35: mol_type = other DNA
aggatcttcaagtttggtggcaaagcttgggattg

SEQ ID NO: 20 - DNA, 24 bp, synthetic construct
  source 1..24: mol_type = other DNA
aaacttgaagatcctggagagtga

SEQ ID NO: 21 - DNA, 35 bp, synthetic construct
  source 1..35: mol_type = other DNA
cgcatctacaaatttggcggaaaaggctgggattg

SEQ ID NO: 22 - DNA, 24 bp, synthetic construct
  source 1..24: mol_type = other DNA
aaatttgtagatgcggttgttcag

SEQ ID NO: 23 - DNA, 35 bp, synthetic construct
  source 1..35: mol_type = other DNA
cgcatctacaaatttggcggaaaagcttgggattg

SEQ ID NO: 24 - DNA, 24 bp, synthetic construct
  source 1..24: mol_type = other DNA
aaatttgtagatgcggttctgaaa

SEQ ID NO: 25 - DNA, 35 bp, synthetic construct
  source 1..35: mol_type = other DNA
aaaatctacaaatttggcggaaaagcttgggattg

SEQ ID NO: 26 - DNA, 24 bp, synthetic construct
  source 1..24: mol_type = other DNA
aaatttgtagattttgttctgcag